European Patent Application EP 4 768 042 A2, published July 1, 2026. Title: NEBULIZATION OF FAB FRAGMENTS. Applicant: ARGENX BV. Application EP. The sequence listing filed with the application follows.

SEQUENCE LISTING (25 sequences)

SEQ ID NO: 1 - protein, 120 aa, synthetic construct
EVQLLESGGGLVQPGGSLRLSCAASGFTFSSYAMSWVRQAPGKGLEWVSAINAGGGSTSYADSVKGRFTISRDNSKNTLYLQMNSLRAEDTAVYYCAKGLRVGVLGFDYWGQGTLVTVSS

SEQ ID NO: 2 - protein, 5 aa, synthetic construct
SYAMS

SEQ ID NO: 3 - protein, 17 aa, synthetic construct
AINAGGGSTSYADSVKG

SEQ ID NO: 4 - protein, 11 aa, synthetic construct
GLRVGVLGFDY

SEQ ID NO: 5 - protein, 106 aa, synthetic construct
SYELTQPLSVSVALGQTARITCDGNNIGSKSAQWYQQKPGQAPVLVIYADEYRPEGIPERFSGSNSGNTATLTISRAQAGDEADYYCQVWDGSAAVFGGGTQLTVL

SEQ ID NO: 6 - protein, 11 aa, synthetic construct
DGNNIGSKSAQ

SEQ ID NO: 7 - protein, 7 aa, synthetic construct
ADEYRPE

SEQ ID NO: 8 - protein, 9 aa, synthetic construct
QVWDGSAAV

SEQ ID NO: 9 - protein, 142 aa, Homo sapiens
MSLLPVPYTEAASLSTGSTVTIKGRPLACFLNEPYLQVDFHTEMKEESDIVFHFQVCFGRRVVMNSREYGAWKQQVESKNMPFQDGQEFELSISVLPDKYQVMVNGQSSYTFDHRIKPEAVKMVQVWRDISLTKFNVSYLKR

SEQ ID NO: 10 - protein, 116 aa, synthetic construct
EVQLLESGGGLVQPGGSLRLSCAASGFTFSSFAMSWVRQAPGKGLEWVSGINSGDGSSVKGRFTISRDNSKNTLYLQMNSLRAEDTAVYYCAKGGATVWGRFHDYWGQGTLVTVSS

SEQ ID NO: 11 - protein, 5 aa, synthetic construct
SFAMS

SEQ ID NO: 12 - protein, 12 aa, synthetic construct
GINSGDGSSVKG

SEQ ID NO: 13 - protein, 12 aa, synthetic construct
GGATVWGRFHDY

SEQ ID NO: 14 - protein, 111 aa, synthetic construct
QSVLTQPPSVSGAPGQRVTISCTGSSSNIGSGSYLSWYQQLPGTAPKLLIYNANNRASGVPDRFSGSKSGTSASLAITGLQAEDEADYYCGCYDSKLSTYVFGGGTKLTVL

SEQ ID NO: 15 - protein, 14 aa, synthetic construct
TGSSSNIGSGSYLS

SEQ ID NO: 16 - protein, 7 aa, synthetic construct
NANNRAS

SEQ ID NO: 17 - protein, 11 aa, synthetic construct
GCYDSKLSTYV

SEQ ID NO: 18 - protein, 119 aa, synthetic construct
EVQLLESGGGLVQPGGSLRLSCAASGFTFRSYDMSWVRQAPGKGLEWVSAIKWHRITYYADSVKGRFTISRDNSKNTLYLQMNSLRAEDTAVYYCATTHGIGTLGFGSWGQGTLVTVSS

SEQ ID NO: 19 - protein, 5 aa, synthetic construct
SYDMS

SEQ ID NO: 20 - protein, 16 aa, synthetic construct
AIKWHRITYYADSVKG

SEQ ID NO: 21 - protein, 11 aa, synthetic construct
THGIGTLGFGS

SEQ ID NO: 22 - protein, 120 aa, synthetic construct
EVQLLESGGGLVQPGGSLRLSCAASGFTFRSYDMSWVRQAPGKGLEWVSAIAQFQHWTYYADSVKGRFTISRDNSKNTLYLQMNSLRAEDTAVYYCATTHGIGTLGFGSWGQGTLVTVSS

SEQ ID NO: 23 - protein, 17 aa, synthetic construct
AIAQFQHWTYYADSVKG

SEQ ID NO: 24 - protein, 120 aa, synthetic construct
EVQLLESGGGLVQPGGSLRLSCAASGFTFSSYAMSWVRQAPGKGLEWVSAINNGGGSTSYADSVKGRFTISRDNSKNTLYLQMNSLRAEDTAVYYCAKGLRVGVLGFDYWGQGTLVTVSS

SEQ ID NO: 25 - protein, 17 aa, synthetic construct
AINNGGGSTSYADSVKG